European Patent Application EP 4 640 711 A1, published October 29, 2025. Title: HIGH-AFFINITY TIGIT ANTIBODY AND USE THEREOF. Applicant: HEFEI TG IMMUNOPHARMA CO., LTD. Application EP 23909713.2, filed November 9, 2023. The sequence listing filed with the application follows.

SEQUENCE LISTING (22 sequences)

SEQ ID NO: 1 - protein, 9 aa, synthetic construct
GSSITSDYA

SEQ ID NO: 2 - protein, 7 aa, synthetic construct
ITYSGRT

SEQ ID NO: 3 - protein, 12 aa, synthetic construct
ARWGLLRRYFDY

SEQ ID NO: 4 - protein, 6 aa, synthetic construct
QDVFNQ

SEQ ID NO: 5 - protein, 7 aa, synthetic construct
SASFRYT

SEQ ID NO: 6 - protein, 9 aa, synthetic construct
QQHYSTPLT

SEQ ID NO: 7 - protein, 119 aa, synthetic construct
QVQLQESGPGLVKPSQTLSLTCTVTGSSITSDYAWNWIRQFPGKKLEWMGYITYSGRTTYNPSLKSRITISRDTSKNQFSLKLSSVTAADTATYYCARWGLLRRYFDYWGQGTLLTVSS

SEQ ID NO: 8 - protein, 107 aa, synthetic construct
DIVMTQSPSSMSTSVGDRVTITCRASQDVFNQVAWYQQKPGKSPKLLIYSASFRYTGVPDRFSGSGSGTDFTFTISSVQAEDFATYYCQQHYSTPLTFGAGTKLELK

SEQ ID NO: 9 - protein, 340 aa, synthetic construct
MMTGTIETTGNISAEKGGSIILQCHLSSTTAQVTQVNWEQQDQLLAICNADLGWHISPSFKDRVAPGPGLGLTLQSLTVNDTGEYFCIYHTYPDGTYTGRIFLEVLELEPKSCDKTHTCPPCPAPELLGGPSVFLFPPKPKDTLMISRTPEVTCVVVDVSHEDPEVKFNWYVDGVEVHNAKTKPREEQYNSTYRVVSVLTVLHQDWLNGKEYKCKVSNKALPAPIEKTISKAKGQPREPQVYTLPPSRDELTKNQVSLTCLVKGFYPSDIAVEWESNGQPENNYKTTPPVLDSDGSFFLYSKLTVDKSRWQQGNVFSCSVMHEALHNHYTQKSLSLSPGK

SEQ ID NO: 10 - protein, 220 aa, synthetic construct
DIVMTQSPDSLAVSLGERATINCKSSQTVLYSSNNKKYLAWYQQKPGQPPNLLIYWASTRESGVPDRFSGSGSGTDFTLTISSLQAEDVAVYYCQQYYSTPFTFGPGTKVEIKRADAAPTVSIFPPSSEQLTSGGASVVCFLNNFYPKDINVKWKIDGSERQNGVLNSWTDQDSKDSTYSMSSTLTLTKDEYERHNSYTCEATHKTSTSPIVKSFNRNEC

SEQ ID NO: 11 - protein, 456 aa, synthetic construct
EVQLQQSGPGLVKPSQTLSLTCAISGDSVSSNSAAWNWIRQSPSRGLEWLGKTYYRFKWYSDYAVSVKGRITINPDTSKNQFSLQLNSVTPEDTAVFYCTRESTTYDLLAGPFDYWGQGTLVTVSSAKTTAPSVYPLAPVCGDTTGSSVTLGCLVKGYFPEPVTLTWNSGSLSSGVHTFPAVLQSDLYTLSSSVTVTSSTWPSQSITCNVAHPASSTKVDKKIEPRGPTIKPCPPCKCPAPNLLGGPSVFIFPPKIKDVLMISLSPIVTCVVVAVSEDDPDVQISWFVNNVEVHTAQTQTHREDYNSTLRVVSALPIQHQDWMSGKEFKCKVNNKDLPAPIERTISKPKGSVRAPQVYVLPPPEEEMTKKQVTLTCMVTDFMPEDIYVEWTNNGKTELNYKNTEPVLDSDGSYFMYSKLRVEKKNWVERNSYSCSVVHEGLHNHHTTKSFSRTPGK

SEQ ID NO: 12 - protein, 216 aa, synthetic construct
EIVLTQSPATLSLSPGERATLSCRASQSVSSYLAWYQQKPGQAPRLLIYDASNRATGIPARFSGSGSGTDFTLTISSLEPEDFAVYYCQQRSNWPPLFTFGPGTKVDIKRADAAPTVSIFPPSSEQLTSGGASVVCFLNNFYPKDINVKWKIDGSERQNGVLNSWTDQDSKDSTYSMSSTLTLTKDEYERHNSYTCEATHKTSTSPIVKSFNRNEC

SEQ ID NO: 13 - protein, 460 aa, synthetic construct
QVQLQESGPGLVKPSETLSLTCTVSGGSVSSGIYYWSWIRQPPGKGLEWIGYIYYSGSTNYNPSLKSRVTISVDTSKNQFSLKLSSVTAADTAVYYCARDYYVSGNYYNVDYYFFGVDVWGQGTTVTVSSAKTTAPSVYPLAPVCGDTTGSSVTLGCLVKGYFPEPVTLTWNSGSLSSGVHTFPAVLQSDLYTLSSSVTVTSSTWPSQSITCNVAHPASSTKVDKKIEPRGPTIKPCPPCKCPAPNLLGGPSVFIFPPKIKDVLMISLSPIVTCVVVAVSEDDPDVQISWFVNNVEVHTAQTQTHREDYNSTLRVVSALPIQHQDWMSGKEFKCKVNNKDLPAPIERTISKPKGSVRAPQVYVLPPPEEEMTKKQVTLTCMVTDFMPEDIYVEWTNNGKTELNYKNTEPVLDSDGSYFMYSKLRVEKKNWVERNSYSCSVVHEGLHNHHTTKSFSRTPGK

SEQ ID NO: 14 - protein, 214 aa, synthetic construct
DIVMTQSPSSMSTSVGDRVTITCRASQDVFNQVAWYQQKPGKSPKLLIYSASFRYTGVPDRFSGSGSGTDFTFTISSVQAEDFATYYCQQHYSTPLTFGAGTKLELKRADAAPTVSIFPPSSEQLTSGGASVVCFLNNFYPKDINVKWKIDGSERQNGVLNSWTDQDSKDSTYSMSSTLTLTKDEYERHNSYTCEATHKTSTSPIVKSFNRNEC

SEQ ID NO: 15 - protein, 449 aa, synthetic construct
QVQLQESGPGLVKPSQTLSLTCTVTGSSITSDYAWNWIRQFPGKKLEWMGYITYSGRTTYNPSLKSRITISRDTSKNQFSLKLSSVTAADTATYYCARWGLLRRYFDYWGQGTLLTVSSAKTTAPSVYPLAPVCGDTTGSSVTLGCLVKGYFPEPVTLTWNSGSLSSGVHTFPAVLQSDLYTLSSSVTVTSSTWPSQSITCNVAHPASSTKVDKKIEPRGPTIKPCPPCKCPAPNLLGGPSVFIFPPKIKDVLMISLSPIVTCVVVDVSEDDPDVQISWFVNNVEVHTAQTQTHREDYNSTLRVVSALPIQHQDWMSGKEFKCKVNNKDLPAPIERTISKPKGSVRAPQVYVLPPPEEEMTKKQVTLTCMVTDFMPEDIYVEWTNNGKTELNYKNTEPVLDSDGSYFMYSKLRVEKKNWVERNSYSCSVVHEGLHNHHTTKSFSRTPGK

SEQ ID NO: 16 - protein, 449 aa, synthetic construct
QVQLQESGPGLVKPSQTLSLTCTVTGSSITSDYAWNWIRQFPGKKLEWMGYITYSGRTTYNPSLKSRITISRDTSKNQFSLKLSSVTAADTATYYCARWGLLRRYFDYWGQGTLLTVSSAKTTAPSVYPLAPVCGDTTGSSVTLGCLVKGYFPEPVTLTWNSGSLSSGVHTFPAVLQSDLYTLSSSVTVTSSTWPSQSITCNVAHPASSTKVDKKIEPRGPTIKPCPPCKCPAPNLLGGPSVFIFPPKIKDVLMISLSPIVTCVVVAVSEDDPDVQISWFVNNVEVHTAQTQTHREDYNSTLRVVSALPIQHQDWMSGKEFKCKVNNKDLPAPIERTISKPKGSVRAPQVYVLPPPEEEMTKKQVTLTCMVTDFMPEDIYVEWTNNGKTELNYKNTEPVLDSDGSYFMYSKLRVEKKNWVERNSYSCSVVHEGLHNHHTTKSFSRTPGK

SEQ ID NO: 17 - protein, 214 aa, synthetic construct
DIVMTQSPSSMSTSVGDRVTITCRASQDVFTAVAWYQQKPGKSPKLLIYSASFRYTGVPDRFSGSGSGTDFTFTISSVQAEDFATYYCQQHYSTPLTFGAGTKLELKRTVAAPSVFIFPPSDEQLKSGTASVVCLLNNFYPREAKVQWKVDNALQSGNSQESVTEQDSKDSTYSLSSTLTLSKADYEKHKVYACEVTHQGLSSPVTKSFNRGEC

SEQ ID NO: 18 - protein, 449 aa, synthetic construct
QVQLQESGPGLVKPSQTLSLTCTVTGSSITSDYAWNWIRQFPGKKLEWMGYITYSGRTTYNPSLKSRITISRDTSKNQFSLKLSSVTAADTATYYCARWGLLRRYFDYWGQGTLLTVSSASTKGPSVFPLAPSSKSTSGGTAALGCLVKDYFPEPVTVSWNSGALTSGVHTFPAVLQSSGLYSLSSVVTVPSSSLGTQTYICNVNHKPSNTKVDKKVEPKSCDKTHTCPPCPAPELLGGPSVFLFPPKPKDTLMISRTPEVTCVVVDVSHEDPEVKFNWYVDGVEVHNAKTKPREEQYNSTYRVVSVLTVLHQDWLNGKEYKCKVSNKALPAPIEKTISKAKGQPREPQVYTLPPSREEMTKNQVSLTCLVKGFYPSDIAVEWESNGQPENNYKTTPPVLDSDGSFFLYSKLTVDKSRWQQGNVFSCSVMHEALHNHYTQKSLSLSPGK

SEQ ID NO: 19 - protein, 214 aa, synthetic construct
DIVMTQSPSSMSTSVGDRVTITCRASQDVFNQVAWYQQKPGKSPKLLIYSASFRYTGVPDRFSGSGSGTDFTFTISSVQAEDFATYYCQQHYSTPLTFGAGTKLELKRTVAAPSVFIFPPSDEQLKSGTASVVCLLNNFYPREAKVQWKVDNALQSGNSQESVTEQDSKDSTYSLSSTLTLSKADYEKHKVYACEVTHQGLSSPVTKSFNRGEC

SEQ ID NO: 20 - protein, 449 aa, synthetic construct; identical to SEQ ID NO: 18

SEQ ID NO: 21 - protein, 449 aa, synthetic construct
QVQLQESGPGLVKPSQTLSLTCTVTGSSITSDYAWNWIRQFPGKKLEWMGYITYSGRTTYNPSLKSRITISRDTSKNQFSLKLSSVTAADTATYYCARWGLLRRYFDYWGQGTLLTVSSASTKGPSVFPLAPSSKSTSGGTAALGCLVKDYFPEPVTVSWNSGALTSGVHTFPAVLQSSGLYSLSSVVTVPSSSLGTQTYICNVNHKPSNTKVDKKVEPKSCDKTHTCPPCPAPEAAGGPSVFLFPPKPKDTLMISRTPEVTCVVVDVSHEDPEVKFNWYVDGVEVHNAKTKPREEQYNSTYRVVSVLTVLHQDWLNGKEYKCKVSNKALPAPIEKTISKAKGQPREPQVYTLPPSREEMTKNQVSLTCLVKGFYPSDIAVEWESNGQPENNYKTTPPVLDSDGSFFLYSKLTVDKSRWQQGNVFSCSVMHEALHNHYTQKSLSLSPGK

SEQ ID NO: 22 - protein, 446 aa, synthetic construct
QVQLQESGPGLVKPSQTLSLTCTVTGSSITSDYAWNWIRQFPGKKLEWMGYITYSGRTTYNPSLKSRITISRDTSKNQFSLKLSSVTAADTATYYCARWGLLRRYFDYWGQGTLLTVSSASTKGPSVFPLAPCSRSTSESTAALGCLVKDYFPEPVTVSWNSGALTSGVHTFPAVLQSSGLYSLSSVVTVPSSSLGTKTYTCNVDHKPSNTKVDKRVESKYGPPCPPCPAPEFEGGPSVFLFPPKPKDTLMISRTPEVTCVVVDVSQEDPEVQFNWYVDGVEVHNAKTKPREEQFNSTYRVVSVLTVLHQDWLNGKEYKCKVSNKGLPSSIEKTISKAKGQPREPQVYTLPPSQEEMTKNQVSLTCLVKGFYPSDIAVEWESNGQPENNYKTTPPVLDSDGSFFLYSRLTVDKSRWQEGNVFSCSVMHEALHNHYTQKSLSLSLGK